European Patent Application EP 4 435 106 A1, published September 25, 2024. Title: Novel aptamer and composition for improving cognitive function and anti-aging comprising the aptamer as an active ingredient. Applicant: NEXMOS Co., Ltd. Application WO. The sequence listing filed with the application follows.

SEQUENCE LISTING (7 sequences)

SEQ ID NO: 1 - DNA, 20 bp, synthetic construct
  misc_feature 1..20: note = aptamer
  source 1..20: mol_type = other DNA
gccagtctcgcggtggcggc

SEQ ID NO: 2 - DNA, 32 bp, synthetic construct
  misc_feature 1..32: note = aptamer
  source 1..32: mol_type = other DNA
gtggaggcggtggccagtctcgcggtggcggc

SEQ ID NO: 3 - DNA, 20 bp, synthetic construct
  misc_feature 1..20: note = aptamer
  source 1..20: mol_type = other DNA
gaggcggtggccagtctcat

SEQ ID NO: 4 - DNA, 20 bp, synthetic construct
  misc_feature 1..20: note = aptamer
  source 1..20: mol_type = other DNA
gccgcggcggtggccgcggc

SEQ ID NO: 5 - DNA, 20 bp, synthetic construct
  misc_feature 1..20: note = aptamer
  source 1..20: mol_type = other DNA
ggaggcggtggccagtctca

SEQ ID NO: 6 - DNA, 20 bp, synthetic construct
  misc_feature 1..20: note = aptamer
  source 1..20: mol_type = other DNA
gagctcgcgccggagttctc

SEQ ID NO: 7 - DNA, 20 bp, synthetic construct
  misc_feature 1..20: note = aptamer
  source 1..20: mol_type = other DNA
ggcggtggccagtctcgcgg